European Patent Specification EP 3 237 005 B1, published September 18, 2024. Title: BISPECIFIC TETRAVALENT ANTIBODIES AND METHODS OF MAKIING AND USING THEREOF. Applicant: SystImmune, Inc. The sequence listing filed with the application follows.

SEQUENCE LISTING (138 sequences)

SEQ ID NO: 1 - DNA, 654 bp, artificial sequence
  Synthesized
cagtctgccctgactcagcctgcctccgtgtctgggtctcctggacagtcgatcaccatctcctgcactggaaccagcagtgacgttggtggttataactttgtctcctggtaccaacaacacccaggcaaagcccccaaactcatgatctatgatgtcagtgatcggccctcaggggtgtctgatcgcttctccggctccaagtctggcaacacggcctccctgatcatctctggcctccaggctgacgacgaggctgattattactgcagctcatatgggagcagcagcactcatgtgattttcggcggagggaccaagctgaccgtcctacgtacggtggctgcaccatctgtcttcatcttcccgccatctgatgagcagttgaaatctggaactgcctctgttgtgtgcctgctgaataacttctatcccagagaggccaaagtacagtggaaggtggataacgccctccaatcgggtaactcccaggagagtgtcacagagcaggacagcaaggacagcacctacagcctcagcagcaccctgacgctgagcaaagcagactacgagaaacacaaagtctacgcctgcgaagtcacccatcagggcctgagctcgcccgtcacaaagagcttcaacaggggagagtgt

SEQ ID NO: 2 - DNA, 333 bp, artificial sequence
  Synthesized
cagtctgccctgactcagcctgcctccgtgtctgggtctcctggacagtcgatcaccatctcctgcactggaaccagcagtgacgttggtggttataactttgtctcctggtaccaacaacacccaggcaaagcccccaaactcatgatctatgatgtcagtgatcggccctcaggggtgtctgatcgcttctccggctccaagtctggcaacacggcctccctgatcatctctggcctccaggctgacgacgaggctgattattactgcagctcatatgggagcagcagcactcatgtgattttcggcggagggaccaagctgaccgtccta

SEQ ID NO: 3 - protein, 218 aa, artificial sequence
  Synthesized
QSALTQPASVSGSPGQSITISCTGTSSDVGGYNFVSWYQQHPGKAPKLMIYDVSDRPSGVSDRFSGSKSGNTASLIISGLQADDEADYYCSSYGSSSTHVIFGGGTKLTVLRTVAAPSVFIFPPSDEQLKSGTASVVCLLNNFYPREAKVQWKVDNALQSGNSQESVTEQDSKDSTYSLSSTLTLSKADYEKHKVYACEVTHQGLSSPVTKSFNRGEC

SEQ ID NO: 4 - protein, 110 aa, artificial sequence
  Synthesized
QSALTQPASVSGSPGQSITISCTGTSSDVGGYNFVSWYQQHPGKAPKLMIYDVSDRPSGVSDRFSGSKSGNTASLIISGLQADDEADYYCSSYGSSSTHVIFGGGTKLTV

SEQ ID NO: 5 - DNA, 1344 bp, artificial sequence
  Synthesized
caggtgcagctgcaggagtcggggggaggcctggtcaagcctggagggtccctgagactctcctgtgcagcctctggattcacctttagtagttattggatgagctgggtccgccaggctccagggaaggggctggagtgggtggccaacataaaccgcgatggaagtgcgagttactatgtggactctgtgaagggccgattcaccatctccagagacgacgccaagaactcactgtatctgcaaatgaacagcctgagagctgaggacacggctgtgtattactgtgcgagagatcgtggggtgggctacttcgatctctggggccgtggcaccctggtcaccgtctcgagcgctagcaccaagggcccatcggtcttccccctggcaccctcctccaagagcacctctgggggcacagcggccctgggctgcctggtcaaggactacttccccgaaccggtgacggtgtcgtggaactcaggcgccctgaccagcggcgtgcacaccttcccggctgtcctacagtcctcaggactctactccctcagcagcgtggtgaccgtgccctccagcagcttgggcacccagacctacatctgcaacgtgaatcacaagcccagcaacaccaaggtggacaagagagttgagcccaaatcttgtgacaaaactcacacatgcccaccgtgcccagcacctgaactcctggggggaccgtcagtcttcctcttccccccaaaacccaaggacaccctcatgatctcccggacccctgaggtcacatgcgtggtggtggacgtgagccacgaagaccctgaggtcaagttcaactggtacgtggacggcgtggaggtgcataatgccaagacaaagccgcgggaggagcagtacaacagcacgtaccgtgtggtcagcgtcctcaccgtcctgcaccaggactggctgaatggcaaggagtacaagtgcaaggtctccaacaaagccctcccagcccccatcgagaaaaccatctccaaagccaaagggcagccccgagaaccacaggtgtacaccctgcccccatcccgggaggagatgaccaagaaccaggtcagcctgacctgcctggtcaaaggcttctatcccagcgacatcgccgtggagtgggagagcaatgggcagccggagaacaactacaagaccacgcctcccgtgctggactccgacggctccttcttcctctatagcaagctcaccgtggacaagagcaggtggcagcaggggaacgtcttctcatgctccgtgatgcatgaggctctgcacaaccactacacgcagaagagcctctccctgtctccgggtaaa

SEQ ID NO: 6 - DNA, 354 bp, artificial sequence
  Synthesized
caggtgcagctgcaggagtcggggggaggcctggtcaagcctggagggtccctgagactctcctgtgcagcctctggattcacctttagtagttattggatgagctgggtccgccaggctccagggaaggggctggagtgggtggccaacataaaccgcgatggaagtgcgagttactatgtggactctgtgaagggccgattcaccatctccagagacgacgccaagaactcactgtatctgcaaatgaacagcctgagagctgaggacacggctgtgtattactgtgcgagagatcgtggggtgggctacttcgatctctggggccgtggcaccctggtcaccgtctcgagc

SEQ ID NO: 7 - protein, 448 aa, artificial sequence
  Synthesized
QVQLQESGGGLVKPGGSLRLSCAASGFTFSSYWMSWVRQAPGKGLEWVANINRDGSASYYVDSVKGRFTISRDDAKNSLYLQMNSLRAEDTAVYYCARDRGVGYFDLWGRGTLVTVSSASTKGPSVFPLAPSSKSTSGGTAALGCLVKDYFPEPVTVSWNSGALTSGVHTFPAVLQSSGLYSLSSVVTVPSSSLGTQTYICNVNHKPSNTKVDKRVEPKSCDKTHTCPPCPAPELLGGPSVFLFPPKPKDTLMISRTPEVTCVVVDVSHEDPEVKFNWYVDGVEVHNAKTKPREEQYNSTYRVVSVLTVLHQDWLNGKEYKCKVSNKALPAPIEKTISKAKGQPREPQVYTLPPSREEMTKNQVSLTCLVKGFYPSDIAVEWESNGQPENNYKTTPPVLDSDGSFFLYSKLTVDKSRWQQGNVFSCSVMHEALHNHYTQKSLSLSPGK

SEQ ID NO: 8 - protein, 118 aa, artificial sequence
  Synthesized
QVQLQESGGGLVKPGGSLRLSCAASGFTFSSYWMSWVRQAPGKGLEWVANINRDGSASYYVDSVKGRFTISRDDAKNSLYLQMNSLRAEDTAVYYCARDRGVGYFDLWGRGTLVTVSS

SEQ ID NO: 9 - DNA, 642 bp, Artificial Sequence
  Synthesized
gacatccagatgacccagtctccatcctccctgtctgcatctgtaggagacagagtcaccatcacttgccaggcgagtcaggacatcagcaactatttaaattggtatcagcagaaaccagggaaagcccctaaactcctgatctacgatgcatccaatttggaaacaggggtcccatcaaggttcagtggaagtggatctgggacagattttactttcaccatcagcagcctgcagcctgaagatattgcaacatatttctgtcaacactttgatcatctcccgctcgctttcggcggagggaccaaggtggaaattaaacgtacggtggctgcaccatctgtcttcatcttcccgccatctgatgagcagttgaaatctggaactgcctctgttgtgtgcctgctgaataacttctatcccagagaggccaaagtacagtggaaggtggataacgccctccaatcgggtaactcccaggagagtgtcacagagcaggacagcaaggacagcacctacagcctcagcagcaccctgacgctgagcaaagcagactacgagaaacacaaagtctacgcctgcgaagtcacccatcagggcctgagctcgcccgtcacaaagagcttcaacaggggagagtgt

SEQ ID NO: 10 - DNA, 321 bp, artificial sequence
  Synthesized
gacatccagatgacccagtctccatcctccctgtctgcatctgtaggagacagagtcaccatcacttgccaggcgagtcaggacatcagcaactatttaaattggtatcagcagaaaccagggaaagcccctaaactcctgatctacgatgcatccaatttggaaacaggggtcccatcaaggttcagtggaagtggatctgggacagattttactttcaccatcagcagcctgcagcctgaagatattgcaacatatttctgtcaacactttgatcatctcccgctcgctttcggcggagggaccaaggtggaaattaaa

SEQ ID NO: 11 - protein, 214 aa, artificial sequence
  Synthesized
DIQMTQSPSSLSASVGDRVTITCQASQDISNYLNWYQQKPGKAPKLLIYDASNLETGVPSRFSGSGSGTDFTFTISSLQPEDIATYFCQHFDHLPLAFGGGTKVEIKRTVAAPSVFIFPPSDEQLKSGTASVVCLLNNFYPREAKVQWKVDNALQSGNSQESVTEQDSKDSTYSLSSTLTLSKADYEKHKVYACEVTHQGLSSPVTKSFNRGEC

SEQ ID NO: 12 - protein, 107 aa, artificial sequence [sequence omitted]

SEQ ID NO: 13 - DNA, 1347 bp, artificial sequence
  Synthesized
caggtgcagctgcaggagtcgggcccaggactggtgaagccttcggagaccctgtccctcacctgcactgtctctggtggctccgtcagcagtggtgattactactggacctggatccggcagtccccagggaagggactggagtggattggacacatctattacagtgggaacaccaattataacccctccctcaagagccgactcaccatatcaattgacacgtccaagactcagttctccctgaagctgagttctgtgaccgctgcggacacggccatttattactgtgtgcgagatcgagtgactggtgcttttgatatctggggccaagggacaatggtcaccgtctcgagcgctagcaccaagggcccatcggtcttccccctggcaccctcctccaagagcacctctgggggcacagcggccctgggctgcctggtcaaggactacttccccgaaccggtgacggtgtcgtggaactcaggcgccctgaccagcggcgtgcacaccttcccggctgtcctacagtcctcaggactctactccctcagcagcgtggtgaccgtgccctccagcagcttgggcacccagacctacatctgcaacgtgaatcacaagcccagcaacaccaaggtggacaagagagttgagcccaaatcttgtgacaaaactcacacatgcccaccgtgcccagcacctgaactcctggggggaccgtcagtcttcctcttccccccaaaacccaaggacaccctcatgatctcccggacccctgaggtcacatgcgtggtggtggacgtgagccacgaagaccctgaggtcaagttcaactggtacgtggacggcgtggaggtgcataatgccaagacaaagccgcgggaggagcagtacaacagcacgtaccgtgtggtcagcgtcctcaccgtcctgcaccaggactggctgaatggcaaggagtacaagtgcaaggtctccaacaaagccctcccagcccccatcgagaaaaccatctccaaagccaaagggcagccccgagaaccacaggtgtacaccctgcccccatcccgggaggagatgaccaagaaccaggtcagcctgacctgcctggtcaaaggcttctatcccagcgacatcgccgtggagtgggagagcaatgggcagccggagaacaactacaagaccacgcctcccgtgctggactccgacggctccttcttcctctatagcaagctcaccgtggacaagagcaggtggcagcaggggaacgtcttctcatgctccgtgatgcatgaggctctgcacaaccactacacgcagaagagcctctccctgtctccgggtaaa

SEQ ID NO: 14 - DNA, 357 bp, artificial sequence
  Synthesized
caggtgcagctgcaggagtcgggcccaggactggtgaagccttcggagaccctgtccctcacctgcactgtctctggtggctccgtcagcagtggtgattactactggacctggatccggcagtccccagggaagggactggagtggattggacacatctattacagtgggaacaccaattataacccctccctcaagagccgactcaccatatcaattgacacgtccaagactcagttctccctgaagctgagttctgtgaccgctgcggacacggccatttattactgtgtgcgagatcgagtgactggtgcttttgatatctggggccaagggacaatggtcaccgtctcgagc

SEQ ID NO: 15 - protein, 449 aa, artificial sequence
  Synthesized
QVQLQESGPGLVKPSETLSLTCTVSGGSVSSGDYYWTWIRQSPGKGLEWIGHIYYSGNTNYNPSLKSRLTISIDTSKTQFSLKLSSVTAADTAIYYCVRDRVTGAFDIWGQGTMVTVSSASTKGPSVFPLAPSSKSTSGGTAALGCLVKDYFPEPVTVSWNSGALTSGVHTFPAVLQSSGLYSLSSVVTVPSSSLGTQTYICNVNHKPSNTKVDKRVEPKSCDKTHTCPPCPAPELLGGPSVFLFPPKPKDTLMISRTPEVTCVVVDVSHEDPEVKFNWYVDGVEVHNAKTKPREEQYNSTYRVVSVLTVLHQDWLNGKEYKCKVSNKALPAPIEKTISKAKGQPREPQVYTLPPSREEMTKNQVSLTCLVKGFYPSDIAVEWESNGQPENNYKTTPPVLDSDGSFFLYSKLTVDKSRWQQGNVFSCSVMHEALHNHYTQKSLSLSPGK

SEQ ID NO: 16 - protein, 119 aa, artificial sequence [sequence omitted]

SEQ ID NO: 17 - DNA, 642 bp, artificial sequence
  Synthesized
gatatccagatgacccagtccccgagctccctgtccgcctctgtgggcgatagggtcaccatcacctgccgtgccagtcagaatattgctactgatgtagcctggtatcaacagaaaccaggaaaagctccgaagcttctgatttactcggcatccttcctctactctggagtcccttctcgcttctctggtagcggttccgggacggatttcactctgaccatcagcagtctgcagccggaagacttcgcaacttattactgtcagcaaagtgagccggagccgtacacgttcggacagggtaccaaggtggagatcaaacgtacggtggctgcaccatctgtcttcatcttcccgccatctgatgagcagttgaaatctggaactgcctctgttgtgtgcctgctgaataacttctatcccagagaggccaaagtacagtggaaggtggataacgccctccaatcgggtaactcccaggagagtgtcacagagcaggacagcaaggacagcacctacagcctcagcagcaccctgacgctgagcaaagcagactacgagaaacacaaagtctacgcctgcgaagtcacccatcagggcctgagctcgcccgtcacaaagagcttcaacaggggagagtgt

SEQ ID NO: 18 - DNA, 321 bp, artificial sequence
  Synthesized
gatatccagatgacccagtccccgagctccctgtccgcctctgtgggcgatagggtcaccatcacctgccgtgccagtcagaatattgctactgatgtagcctggtatcaacagaaaccaggaaaagctccgaagcttctgatttactcggcatccttcctctactctggagtcccttctcgcttctctggtagcggttccgggacggatttcactctgaccatcagcagtctgcagccggaagacttcgcaacttattactgtcagcaaagtgagccggagccgtacacgttcggacagggtaccaaggtggagatcaaa

SEQ ID NO: 19 - protein, 214 aa, artificial sequence
  Synthesized
DIQMTQSPSSLSASVGDRVTITCRASQNIATDVAWYQQKPGKAPKLLIYSASFLYSGVPSRFSGSGSGTDFTLTISSLQPEDFATYYCQQSEPEPYTFGQGTKVEIKRTVAAPSVFIFPPSDEQLKSGTASVVCLLNNFYPREAKVQWKVDNALQSGNSQESVTEQDSKDSTYSLSSTLTLSKADYEKHKVYACEVTHQGLSSPVTKSFNRGEC

SEQ ID NO: 20 - protein, 107 aa, artificial sequence [sequence omitted]

SEQ ID NO: 21 - DNA, 1353 bp, artificial sequence
  Synthesized
gaggtgcagctggtcgagtctggcggcggactggtgcagcccggtggctctctgcgactgtcttgtgccgcctctggcttcaccctcagtggcgattggatccactgggtgcgacaggctcccggaaagggcctggagtgggtgggtgagatctctgctgccggtggctacaccgattacgccgactctgtgaagggccgattcaccatctctgccgacacctctaagaacaccgcctacctgcagatgaactctctgcgagccgaggacaccgctgtgtactactgtgcacgagaaagtagagtttccttcgaagccgccatggactactggggccagggcaccctggtgaccgtgtcctctgctagcaccaagggcccatcggtcttccccctggcaccctcctccaagagcacctctgggggcacagcggccctgggctgcctggtcaaggactacttccccgaaccggtgacggtgtcgtggaactcaggcgccctgaccagcggcgtgcacaccttcccggctgtcctacagtcctcaggactctactccctcagcagcgtggtgaccgtgccctccagcagcttgggcacccagacctacatctgcaacgtgaatcacaagcccagcaacaccaaggtggacaagagagttgagcccaaatcttgtgacaaaactcacacatgcccaccgtgcccagcacctgaactcctggggggaccgtcagtcttcctcttccccccaaaacccaaggacaccctcatgatctcccggacccctgaggtcacatgcgtggtggtggacgtgagccacgaagaccctgaggtcaagttcaactggtacgtggacggcgtggaggtgcataatgccaagacaaagccgcgggaggagcagtacaacagcacgtaccgtgtggtcagcgtcctcaccgtcctgcaccaggactggctgaatggcaaggagtacaagtgcaaggtctccaacaaagccctcccagcccccatcgagaaaaccatctccaaagccaaagggcagccccgagaaccacaggtgtacaccctgcccccatcccgggaggagatgaccaagaaccaggtcagcctgacctgcctggtcaaaggcttctatcccagcgacatcgccgtggagtgggagagcaatgggcagccggagaacaactacaagaccacgcctcccgtgctggactccgacggctccttcttcctctatagcaagctcaccgtggacaagagcaggtggcagcaggggaacgtcttctcatgctccgtgatgcatgaggctctgcacaaccactacacgcagaagagcctctccctgtctccgggtaaa

SEQ ID NO: 22 - DNA, 363 bp, Artificial Sequence
  Synthesized
gaggtgcagctggtcgagtctggcggcggactggtgcagcccggtggctctctgcgactgtcttgtgccgcctctggcttcaccctcagtggcgattggatccactgggtgcgacaggctcccggaaagggcctggagtgggtgggtgagatctctgctgccggtggctacaccgattacgccgactctgtgaagggccgattcaccatctctgccgacacctctaagaacaccgcctacctgcagatgaactctctgcgagccgaggacaccgctgtgtactactgtgcacgagaaagtagagtttccttcgaagccgccatggactactggggccagggcaccctggtgaccgtgtcctct

SEQ ID NO: 23 - protein, 451 aa, artificial sequence
  Synthesized
EVQLVESGGGLVQPGGSLRLSCAASGFTLSGDWIHWVRQAPGKGLEWVGEISAAGGYTDYADSVKGRFTISADTSKNTAYLQMNSLRAEDTAVYYCARESRVSFEAAMDYWGQGTLVTVSSASTKGPSVFPLAPSSKSTSGGTAALGCLVKDYFPEPVTVSWNSGALTSGVHTFPAVLQSSGLYSLSSVVTVPSSSLGTQTYICNVNHKPSNTKVDKRVEPKSCDKTHTCPPCPAPELLGGPSVFLFPPKPKDTLMISRTPEVTCVVVDVSHEDPEVKFNWYVDGVEVHNAKTKPREEQYNSTYRVVSVLTVLHQDWLNGKEYKCKVSNKALPAPIEKTISKAKGQPREPQVYTLPPSREEMTKNQVSLTCLVKGFYPSDIAVEWESNGQPENNYKTTPPVLDSDGSFFLYSKLTVDKSRWQQGNVFSCSVMHEALHNHYTQKSLSLSPGK

SEQ ID NO: 24 - protein, 121 aa, artificial sequence [sequence omitted]

SEQ ID NO: 25 - DNA, 657 bp, artificial sequence
  Synthesized
gatattcaaatgactcaatctccttcttctctttctgcttctgttggtgatcgtgttactattacttgtcgttcttctcaaaatattgttcattctaatggtaatacttatcttgattggtatcaacaaactcctggtaaagctcctaaacttcttatttataaagtttctaatcgtttttctggtgttccttctcgtttttctggttctggttctggtactgattttacttttactatttcttctcttcaacctgaagatattgctacttattattgttttcaatattctcatgttccttggacttttggtcaaggtactaaacttcaaattactcgtacggtggctgcaccatctgtcttcatcttcccgccatctgatgagcagttgaaatctggaactgcctctgttgtgtgcctgctgaataacttctatcccagagaggccaaagtacagtggaaggtggataacgccctccaatcgggtaactcccaggagagtgtcacagagcaggacagcaaggacagcacctacagcctcagcagcaccctgacgctgagcaaagcagactacgagaaacacaaagtctacgcctgcgaagtcacccatcagggcctgagctcgcccgtcacaaagagcttcaacaggggagagtgt

SEQ ID NO: 26 - DNA, 336 bp, artificial sequence
  Synthesized
gatattcaaatgactcaatctccttcttctctttctgcttctgttggtgatcgtgttactattacttgtcgttcttctcaaaatattgttcattctaatggtaatacttatcttgattggtatcaacaaactcctggtaaagctcctaaacttcttatttataaagtttctaatcgtttttctggtgttccttctcgtttttctggttctggttctggtactgattttacttttactatttcttctcttcaacctgaagatattgctacttattattgttttcaatattctcatgttccttggacttttggtcaaggtactaaacttcaaattact

SEQ ID NO: 27 - protein, 219 aa, artificial sequence
  Synthesized
DIQMTQSPSSLSASVGDRVTITCRSSQNIVHSNGNTYLDWYQQTPGKAPKLLIYKVSNRFSGVPSRFSGSGSGTDFTFTISSLQPEDIATYYCFQYSHVPWTFGQGTKLQITRTVAAPSVFIFPPSDEQLKSGTASVVCLLNNFYPREAKVQWKVDNALQSGNSQESVTEQDSKDSTYSLSSTLTLSKADYEKHKVYACEVTHQGLSSPVTKSFNRGEC

SEQ ID NO: 28 - protein, 112 aa, artificial sequence [sequence omitted]

SEQ ID NO: 29 - DNA, 1359 bp, artificial sequence
  Synthesized
caagttcaacttcaacaatctggtgctgaagttaaaaaacctggttcttctgttaaagtttcttgtaaagcctctggttatacttttactaattattatatttattgggttcgtcaagctcctggtcaaggtcttgaatggattggtggtattaatcctacttctggtggttctaattttaatgaaaaatttaaaactcgtgttactattactgttgatgaatctacgaacactgcttatatggaactttcttctcttcgttctgaagatactgctttttatttttgtgcgcgtcaaggtctttggtttgattctgatggtcgtggttttgatttttggggtcaaggttccactgttactgtctcgagcgctagcaccaagggcccatcggtcttccccctggcaccctcctccaagagcacctctgggggcacagcggccctgggctgcctggtcaaggactacttccccgaaccggtgacggtgtcgtggaactcaggcgccctgaccagcggcgtgcacaccttcccggctgtcctacagtcctcaggactctactccctcagcagcgtggtgaccgtgccctccagcagcttgggcacccagacctacatctgcaacgtgaatcacaagcccagcaacaccaaggtggacaagagagttgagcccaaatcttgtgacaaaactcacacatgcccaccgtgcccagcacctgaactcctggggggaccgtcagtcttcctcttccccccaaaacccaaggacaccctcatgatctcccggacccctgaggtcacatgcgtggtggtggacgtgagccacgaagaccctgaggtcaagttcaactggtacgtggacggcgtggaggtgcataatgccaagacaaagccgcgggaggagcagtacaacagcacgtaccgtgtggtcagcgtcctcaccgtcctgcaccaggactggctgaatggcaaggagtacaagtgcaaggtctccaacaaagccctcccagcccccatcgagaaaaccatctccaaagccaaagggcagccccgagaaccacaggtgtacaccctgcccccatcccgggaggagatgaccaagaaccaggtcagcctgacctgcctggtcaaaggcttctatcccagcgacatcgccgtggagtgggagagcaatgggcagccggagaacaactacaagaccacgcctcccgtgctggactccgacggctccttcttcctctatagcaagctcaccgtggacaagagcaggtggcagcaggggaacgtcttctcatgctccgtgatgcatgaggctctgcacaaccactacacgcagaagagcctctccctgtctccgggtaaa

SEQ ID NO: 30 - DNA, 369 bp, artificial sequence
  Synthesized
caagttcaacttcaacaatctggtgctgaagttaaaaaacctggttcttctgttaaagtttcttgtaaagcctctggttatacttttactaattattatatttattgggttcgtcaagctcctggtcaaggtcttgaatggattggtggtattaatcctacttctggtggttctaattttaatgaaaaatttaaaactcgtgttactattactgttgatgaatctacgaacactgcttatatggaactttcttctcttcgttctgaagatactgctttttatttttgtgcgcgtcaaggtctttggtttgattctgatggtcgtggttttgatttttggggtcaaggttccactgttactgtctcgagc

SEQ ID NO: 31 - protein, 453 aa, artificial sequence
  Synthesized
QVQLQQSGAEVKKPGSSVKVSCKASGYTFTNYYIYWVRQAPGQGLEWIGGINPTSGGSNFNEKFKTRVTITVDESTNTAYMELSSLRSEDTAFYFCARQGLWFDSDGRGFDFWGQGSTVTVSSASTKGPSVFPLAPSSKSTSGGTAALGCLVKDYFPEPVTVSWNSGALTSGVHTFPAVLQSSGLYSLSSVVTVPSSSLGTQTYICNVNHKPSNTKVDKRVEPKSCDKTHTCPPCPAPELLGGPSVFLFPPKPKDTLMISRTPEVTCVVVDVSHEDPEVKFNWYVDGVEVHNAKTKPREEQYNSTYRVVSVLTVLHQDWLNGKEYKCKVSNKALPAPIEKTISKAKGQPREPQVYTLPPSREEMTKNQVSLTCLVKGFYPSDIAVEWESNGQPENNYKTTPPVLDSDGSFFLYSKLTVDKSRWQQGNVFSCSVMHEALHNHYTQKSLSLSPGK

SEQ ID NO: 32 - protein, 123 aa, artificial sequence
  Synthesized
QVQLQQSGAEVKKPGSSVKVSCKASGYTFTNYYIYWVRQAPGQGLEWIGGINPTSGGSNFNEKFKTRVTITVDESTNTAYMELSSLRSEDTAFYFCARQGLWFDSDGRGFDFWGQGSTVTVSS

SEQ ID NO: 33 - DNA, 657 bp, artificial sequence; identical to SEQ ID NO: 25
  Synthesized

SEQ ID NO: 34 - DNA, 336 bp, artificial sequence; identical to SEQ ID NO: 26
  Synthesized

SEQ ID NO: 35 - protein, 218 aa, artificial sequence; identical to SEQ ID NO: 3
  Synthesized

SEQ ID NO: 36 - protein, 111 aa, artificial sequence
  Synthesized
QSALTQPASVSGSPGQSITISCTGTSSDVGGYNFVSWYQQHPGKAPKLMIYDVSDRPSGVSDRFSGSKSGNTASLIISGLQADDEADYYCSSYGSSSTHVIFGGGTKLTVL

SEQ ID NO: 37 - DNA, 1356 bp, artificial sequence
  Synthesized
caggtgcagctgcagcagagcggcgccgaggtgaagaagcccggcagcagcgtgaaggtgagctgcaaggccagcggctacaccttcaccaactactacatctactgggtgcggcaggcccccggccagggcctggagtggatcggcggcatcaaccccaccagcggcggcagcaacttcaacgagaagttcaagacccgggtgaccatcaccgccgacgagagcagcaccaccgcctacatggagctgagcagcctgcggagcgaggacaccgccttctacttctgcacccggcagggcctgtggttcgacagcgacggccggggcttcgacttctggggccagggcaccaccgtgaccgtgagcagcgctagcaccaagggcccatcggtcttccccctggcaccctcctccaagagcacctctgggggcacagcggccctgggctgcctggtcaaggactacttccccgaaccggtgacggtgtcgtggaactcaggcgccctgaccagcggcgtgcacaccttcccggctgtcctacagtcctcaggactctactccctcagcagcgtggtgaccgtgccctccagcagcttgggcacccagacctacatctgcaacgtgaatcacaagcccagcaacaccaaggtggacaagagagttgagcccaaatcttgtgacaaaactcacacatgcccaccgtgcccagcacctgaactcctggggggaccgtcagtcttcctcttccccccaaaacccaaggacaccctcatgatctcccggacccctgaggtcacatgcgtggtggtggacgtgagccacgaagaccctgaggtcaagttcaactggtacgtggacggcgtggaggtgcataatgccaagacaaagccgcgggaggagcagtacaacagcacgtaccgtgtggtcagcgtcctcaccgtcctgcaccaggactggctgaatggcaaggagtacaagtgcaaggtctccaacaaagccctcccagcccccatcgagaaaaccatctccaaagccaaagggcagccccgagaaccacaggtgtacaccctgcccccatcccgggatgagctgaccaagaaccaggtcagcctgacctgcctggtcaaaggcttctatcccagcgacatcgccgtggagtgggagagcaatgggcagccggagaacaactacaagaccacgcctcccgtgctggactccgacggctccttcttcctctatagcaagctcaccgtggacaagagcaggtggcagcaggggaacgtcttctcatgctccgtgatgcatgaggctctgcacaaccactacacgcagaagagcctctccctgtctccgggt

SEQ ID NO: 38 - DNA, 369 bp, artificial sequence
  Synthesized
caggtgcagctgcagcagagcggcgccgaggtgaagaagcccggcagcagcgtgaaggtgagctgcaaggccagcggctacaccttcaccaactactacatctactgggtgcggcaggcccccggccagggcctggagtggatcggcggcatcaaccccaccagcggcggcagcaacttcaacgagaagttcaagacccgggtgaccatcaccgccgacgagagcagcaccaccgcctacatggagctgagcagcctgcggagcgaggacaccgccttctacttctgcacccggcagggcctgtggttcgacagcgacggccggggcttcgacttctggggccagggcaccaccgtgaccgtgagcagc

SEQ ID NO: 39 - protein, 452 aa, artificial sequence
  Synthesized
QVQLQQSGAEVKKPGSSVKVSCKASGYTFTNYYIYWVRQAPGQGLEWIGGINPTSGGSNFNEKFKTRVTITADESSTTAYMELSSLRSEDTAFYFCTRQGLWFDSDGRGFDFWGQGTTVTVSSASTKGPSVFPLAPSSKSTSGGTAALGCLVKDYFPEPVTVSWNSGALTSGVHTFPAVLQSSGLYSLSSVVTVPSSSLGTQTYICNVNHKPSNTKVDKRVEPKSCDKTHTCPPCPAPELLGGPSVFLFPPKPKDTLMISRTPEVTCVVVDVSHEDPEVKFNWYVDGVEVHNAKTKPREEQYNSTYRVVSVLTVLHQDWLNGKEYKCKVSNKALPAPIEKTISKAKGQPREPQVYTLPPSRDELTKNQVSLTCLVKGFYPSDIAVEWESNGQPENNYKTTPPVLDSDGSFFLYSKLTVDKSRWQQGNVFSCSVMHEALHNHYTQKSLSLSPG

SEQ ID NO: 40 - protein, 123 aa, artificial sequence [sequence omitted]

SEQ ID NO: 41 - DNA, 642 bp, artificial sequence
  Synthesized
gacatcttgctgactcagtctccagtcatcctgtctgtgagtccaggagaaagagtcagtttctcctgcagggccagtcagagtattggcacaaacatacactggtatcagcaaagaacaaatggttctccaaggcttctcataaagtatgcttctgagtctatctctgggattccttccaggtttagtggcagtggatcagggacagattttactcttagcatcaacagtgtggagtctgaagatattgcagattattactgtcaacaaaataataactggccaaccacgttcggtgctgggaccaagctggagctgaaacgtacggtggctgcaccatctgtcttcatcttcccgccatctgatgagcagttgaaatctggaactgcctctgttgtgtgcctgctgaataacttctatcccagagaggccaaagtacagtggaaggtggataacgccctccaatcgggtaactcccaggagagtgtcacagagcaggacagcaaggacagcacctacagcctcagcagcaccctgacgctgagcaaagcagactacgagaaacacaaagtctacgcctgcgaagtcacccatcagggcctgagctcgcccgtcacaaagagcttcaacaggggagagtgt

SEQ ID NO: 42 - DNA, 321 bp, artificial sequence
  Synthesized
gacatcttgctgactcagtctccagtcatcctgtctgtgagtccaggagaaagagtcagtttctcctgcagggccagtcagagtattggcacaaacatacactggtatcagcaaagaacaaatggttctccaaggcttctcataaagtatgcttctgagtctatctctgggattccttccaggtttagtggcagtggatcagggacagattttactcttagcatcaacagtgtggagtctgaagatattgcagattattactgtcaacaaaataataactggccaaccacgttcggtgctgggaccaagctggagctgaaa

SEQ ID NO: 43 - protein, 214 aa, artificial sequence
  Synthesized
DILLTQSPVILSVSPGERVSFSCRASQSIGTNIHWYQQRTNGSPRLLIKYASESISGIPSRFSGSGSGTDFTLSINSVESEDIADYYCQQNNNWPTTFGAGTKLELKRTVAAPSVFIFPPSDEQLKSGTASVVCLLNNFYPREAKVQWKVDNALQSGNSQESVTEQDSKDSTYSLSSTLTLSKADYEKHKVYACEVTHQGLSSPVTKSFNRGEC

SEQ ID NO: 44 - protein, 107 aa, artificial sequence
  Synthesized
DILLTQSPVILSVSPGERVSFSCRASQSIGTNIHWYQQRTNGSPRLLIKYASESISGIPSRFSGSGSGTDFTLSINSVESEDIADYYCQQNNNWPTTFGAGTKLELK

SEQ ID NO: 45 - DNA, 1347 bp, artificial sequence
  Synthesized
caggtgcagctgaagcagtcaggacctggcctagtgcagccctcacagagcctgtccatcacctgcacagtctctggtttctcattaactaactatggtgtacactgggttcgccagtctccaggaaagggtctggagtggctgggagtgatatggagtggtggaaacacagactataatacacctttcacatccagactgagcatcaacaaggacaattccaagagccaagttttctttaaaatgaacagtctgcaatctaatgacacagccatatattactgtgccagagccctcacctactatgattacgagtttgcttactggggccaagggactctggtcactgtctctagcgctagcaccaagggcccatcggtcttccccctggcaccctcctccaagagcacctctgggggcacagcggccctgggctgcctggtcaaggactacttccccgaaccggtgacggtgtcgtggaactcaggcgccctgaccagcggcgtgcacaccttcccggctgtcctacagtcctcaggactctactccctcagcagcgtggtgaccgtgccctccagcagcttgggcacccagacctacatctgcaacgtgaatcacaagcccagcaacaccaaggtggacaagagagttgagcccaaatcttgtgacaaaactcacacatgcccaccgtgcccagcacctgaactcctggggggaccgtcagtcttcctcttccccccaaaacccaaggacaccctcatgatctcccggacccctgaggtcacatgcgtggtggtggacgtgagccacgaagaccctgaggtcaagttcaactggtacgtggacggcgtggaggtgcataatgccaagacaaagccgcgggaggagcagtacaacagcacgtaccgtgtggtcagcgtcctcaccgtcctgcaccaggactggctgaatggcaaggagtacaagtgcaaggtctccaacaaagccctcccagcccccatcgagaaaaccatctccaaagccaaagggcagccccgagaaccacaggtgtacaccctgcccccatcccgggaggagatgaccaagaaccaggtcagcctgacctgcctggtcaaaggcttctatcccagcgacatcgccgtggagtgggagagcaatgggcagccggagaacaactacaagaccacgcctcccgtgctggactccgacggctccttcttcctctatagcaagctcaccgtggacaagagcaggtggcagcaggggaacgtcttctcatgctccgtgatgcatgaggctctgcacaaccactacacgcagaagagcctctccctgtctccgggtaaa

SEQ ID NO: 46 - DNA, 357 bp, artificial sequence
  Synthesized
caggtgcagctgaagcagtcaggacctggcctagtgcagccctcacagagcctgtccatcacctgcacagtctctggtttctcattaactaactatggtgtacactgggttcgccagtctccaggaaagggtctggagtggctgggagtgatatggagtggtggaaacacagactataatacacctttcacatccagactgagcatcaacaaggacaattccaagagccaagttttctttaaaatgaacagtctgcaatctaatgacacagccatatattactgtgccagagccctcacctactatgattacgagtttgcttactggggccaagggactctggtcactgtctctagc

SEQ ID NO: 47 - protein, 449 aa, artificial sequence
  Synthesized
QVQLKQSGPGLVQPSQSLSITCTVSGFSLTNYGVHWVRQSPGKGLEWLGVIWSGGNTDYNTPFTSRLSINKDNSKSQVFFKMNSLQSNDTAIYYCARALTYYDYEFAYWGQGTLVTVSSASTKGPSVFPLAPSSKSTSGGTAALGCLVKDYFPEPVTVSWNSGALTSGVHTFPAVLQSSGLYSLSSVVTVPSSSLGTQTYICNVNHKPSNTKVDKRVEPKSCDKTHTCPPCPAPELLGGPSVFLFPPKPKDTLMISRTPEVTCVVVDVSHEDPEVKFNWYVDGVEVHNAKTKPREEQYNSTYRVVSVLTVLHQDWLNGKEYKCKVSNKALPAPIEKTISKAKGQPREPQVYTLPPSREEMTKNQVSLTCLVKGFYPSDIAVEWESNGQPENNYKTTPPVLDSDGSFFLYSKLTVDKSRWQQGNVFSCSVMHEALHNHYTQKSLSLSPGK

SEQ ID NO: 48 - protein, 119 aa, artificial sequence
  Synthesized
QVQLKQSGPGLVQPSQSLSITCTVSGFSLTNYGVHWVRQSPGKGLEWLGVIWSGGNTDYNTPFTSRLSINKDNSKSQVFFKMNSLQSNDTAIYYCARALTYYDYEFAYWGQGTLVTVSS

SEQ ID NO: 49 - DNA, 654 bp, artificial sequence; identical to SEQ ID NO: 1
  Synthesized

SEQ ID NO: 50 - DNA, 333 bp, artificial sequence; identical to SEQ ID NO: 2
  Synthesized

SEQ ID NO: 51 - protein, 218 aa, artificial sequence; identical to SEQ ID NO: 3
  Synthesized

SEQ ID NO: 52 - protein, 111 aa, artificial sequence; identical to SEQ ID NO: 36
  Synthesized

SEQ ID NO: 53 - DNA, 2100 bp, artificial sequence
  Synthesized
caggtgcagctgcaggagtcggggggaggcctggtcaagcctggagggtccctgagactctcctgtgcagcctctggattcacctttagtagttattggatgagctgggtccgccaggctccagggaaggggctggagtgggtggccaacataaaccgcgatggaagtgcgagttactatgtggactctgtgaagggccgattcaccatctccagagacgacgccaagaactcactgtatctgcaaatgaacagcctgagagctgaggacacggctgtgtattactgtgcgagagatcgtggggtgggctacttcgatctctggggccgtggcaccctggtcaccgtctcgagcgctagcaccaagggcccatcggtcttccccctggcaccctcctccaagagcacctctgggggcacagcggccctgggctgcctggtcaaggactacttccccgaaccggtgacggtgtcgtggaactcaggcgccctgaccagcggcgtgcacaccttcccggctgtcctacagtcctcaggactctactccctcagcagcgtggtgaccgtgccctccagcagcttgggcacccagacctacatctgcaacgtgaatcacaagcccagcaacaccaaggtggacaagagagttgagcccaaatcttgtgacaaaactcacacatgcccaccgtgcccagcacctgaactcctggggggaccgtcagtcttcctcttccccccaaaacccaaggacaccctcatgatctcccggacccctgaggtcacatgcgtggtggtggacgtgagccacgaagaccctgaggtcaagttcaactggtacgtggacggcgtggaggtgcataatgccaagacaaagccgcgggaggagcagtacaacagcacgtaccgtgtggtcagcgtcctcaccgtcctgcaccaggactggctgaatggcaaggagtacaagtgcaaggtctccaacaaagccctcccagcccccatcgagaaaaccatctccaaagccaaagggcagccccgagaaccacaggtgtacaccctgcccccatcccgggaggagatgaccaagaaccaggtcagcctgacctgcctggtcaaaggcttctatcccagcgacatcgccgtggagtgggagagcaatgggcagccggagaacaactacaagaccacgcctcccgtgctggactccgacggctccttcttcctctatagcaagctcaccgtggacaagagcaggtggcagcaggggaacgtcttctcatgctccgtgatgcatgaggctctgcacaaccactacacgcagaagagcctctccctgtctccgggtaaaggcggtggaggatccggcggtggtggatcacaggtgcagctgcaggagtcgggcccaggactggtgaagccttcggagaccctgtccctcacctgcactgtctctggtggctccgtcagcagtggtgattactactggacctggatacggcagtccccagggaagggactggagtggattggacacatctattacagtgggaacaccaattataacccctccctcaagagccgactcaccatatcaattgacacgtccaagactcagttctccctgaagctgagttctgtgaccgctgcggacacggccatttattactgtgtgcgagatcgagtgactggtgcttttgatatctggggccaagggacaatggtcaccgtctcgagcggtggaggcggttcaggcggaggtggttccggcggtggcggctccgacatccagatgacccagtctccatcctccctgtctgcatctgtaggagacagagtcaccatcacttgccaggcgagtcaggacatcagcaactatttaaattggtatcagcagaaaccagggaaagcccctaaactcctgatctacgatgcatccaatttggaaacaggggtcccatcaaggttcagtggaagtggatctgggacagattttactttcaccatcagcagcctgcagcctgaagatattgcaacatatttctgtcaacactttgatcatctcccgctcgctttcggcggagggaccaaggtggaaattaaacgt

SEQ ID NO: 54 - DNA, 354 bp, artificial sequence; identical to SEQ ID NO: 6
  Synthesized

SEQ ID NO: 55 - DNA, 726 bp, artificial sequence
  Synthesized
caggtgcagctgcaggagtcgggcccaggactggtgaagccttcggagaccctgtccctcacctgcactgtctctggtggctccgtcagcagtggtgattactactggacctggatacggcagtccccagggaagggactggagtggattggacacatctattacagtgggaacaccaattataacccctccctcaagagccgactcaccatatcaattgacacgtccaagactcagttctccctgaagctgagttctgtgaccgctgcggacacggccatttattactgtgtgcgagatcgagtgactggtgcttttgatatctggggccaagggacaatggtcaccgtctcgagcggtggaggcggttcaggcggaggtggttccggcggtggcggctccgacatccagatgacccagtctccatcctccctgtctgcatctgtaggagacagagtcaccatcacttgccaggcgagtcaggacatcagcaactatttaaattggtatcagcagaaaccagggaaagcccctaaactcctgatctacgatgcatccaatttggaaacaggggtcccatcaaggttcagtggaagtggatctgggacagattttactttcaccatcagcagcctgcagcctgaagatattgcaacatatttctgtcaacactttgatcatctcccgctcgctttcggcggagggaccaaggtggaaattaaacgt

SEQ ID NO: 56 - protein, 700 aa, artificial sequence
  Synthesized
QVQLQESGGGLVKPGGSLRLSCAASGFTFSSYWMSWVRQAPGKGLEWVANINRDGSASYYVDSVKGRFTISRDDAKNSLYLQMNSLRAEDTAVYYCARDRGVGYFDLWGRGTLVTVSSASTKGPSVFPLAPSSKSTSGGTAALGCLVKDYFPEPVTVSWNSGALTSGVHTFPAVLQSSGLYSLSSVVTVPSSSLGTQTYICNVNHKPSNTKVDKRVEPKSCDKTHTCPPCPAPELLGGPSVFLFPPKPKDTLMISRTPEVTCVVVDVSHEDPEVKFNWYVDGVEVHNAKTKPREEQYNSTYRVVSVLTVLHQDWLNGKEYKCKVSNKALPAPIEKTISKAKGQPREPQVYTLPPSREEMTKNQVSLTCLVKGFYPSDIAVEWESNGQPENNYKTTPPVLDSDGSFFLYSKLTVDKSRWQQGNVFSCSVMHEALHNHYTQKSLSLSPGKGGGGSGGGGSQVQLQESGPGLVKPSETLSLTCTVSGGSVSSGDYYWTWIRQSPGKGLEWIGHIYYSGNTNYNPSLKSRLTISIDTSKTQFSLKLSSVTAADTAIYYCVRDRVTGAFDIWGQGTMVTVSSGGGGSGGGGSGGGGSDIQMTQSPSSLSASVGDRVTITCQASQDISNYLNWYQQKPGKAPKLLIYDASNLETGVPSRFSGSGSGTDFTFTISSLQPEDIATYFCQHFDHLPLAFGGGTKVEIKR

SEQ ID NO: 57 - protein, 118 aa, artificial sequence; identical to SEQ ID NO: 8
  Synthesized

SEQ ID NO: 58 - protein, 242 aa, artificial sequence
  Synthesized
QVQLQESGPGLVKPSETLSLTCTVSGGSVSSGDYYWTWIRQSPGKGLEWIGHIYYSGNTNYNPSLKSRLTISIDTSKTQFSLKLSSVTAADTAIYYCVRDRVTGAFDIWGQGTMVTVSSGGGGSGGGGSGGGGSDIQMTQSPSSLSASVGDRVTITCQASQDISNYLNWYQQKPGKAPKLLIYDASNLETGVPSRFSGSGSGTDFTFTISSLQPEDIATYFCQHFDHLPLAFGGGTKVEIKR

SEQ ID NO: 59 - DNA, 642 bp, artificial sequence; identical to SEQ ID NO: 9
  Synthesized

SEQ ID NO: 60 - DNA, 321 bp, artificial sequence; identical to SEQ ID NO: 10
  Synthesized

SEQ ID NO: 61 - protein, 214 aa, artificial sequence; identical to SEQ ID NO: 11
  Synthesized

SEQ ID NO: 62 - protein, 107 aa, artificial sequence [sequence omitted]

SEQ ID NO: 63 - DNA, 2109 bp, artificial sequence
  Synthesized
caggtgcagctgcaggagtcgggcccaggactggtgaagccttcggagaccctgtccctcacctgcactgtctctggtggctccgtcagcagtggtgattactactggacctggatccggcagtccccagggaagggactggagtggattggacacatctattacagtgggaacaccaattataacccctccctcaagagccgactcaccatatcaattgacacgtccaagactcagttctccctgaagctgagttctgtgaccgctgcggacacggccatttattactgtgtgcgagatcgagtgactggtgcttttgatatctggggccaagggacaatggtcaccgtctcgagcgctagcaccaagggcccatcggtcttccccctggcaccctcctccaagagcacctctgggggcacagcggccctgggctgcctggtcaaggactacttccccgaaccggtgacggtgtcgtggaactcaggcgccctgaccagcggcgtgcacaccttcccggctgtcctacagtcctcaggactctactccctcagcagcgtggtgaccgtgccctccagcagcttgggcacccagacctacatctgcaacgtgaatcacaagcccagcaacaccaaggtggacaagagagttgagcccaaatcttgtgacaaaactcacacatgcccaccgtgcccagcacctgaactcctggggggaccgtcagtcttcctcttccccccaaaacccaaggacaccctcatgatctcccggacccctgaggtcacatgcgtggtggtggacgtgagccacgaagaccctgaggtcaagttcaactggtacgtggacggcgtggaggtgcataatgccaagacaaagccgcgggaggagcagtacaacagcacgtaccgtgtggtcagcgtcctcaccgtcctgcaccaggactggctgaatggcaaggagtacaagtgcaaggtctccaacaaagccctcccagcccccatcgagaaaaccatctccaaagccaaagggcagccccgagaaccacaggtgtacaccctgcccccatcccgggaggagatgaccaagaaccaggtcagcctgacctgcctggtcaaaggcttctatcccagcgacatcgccgtggagtgggagagcaatgggcagccggagaacaactacaagaccacgcctcccgtgctggactccgacggctccttcttcctctatagcaagctcaccgtggacaagagcaggtggcagcaggggaacgtcttctcatgctccgtgatgcatgaggctctgcacaaccactacacgcagaagagcctctccctgtctccgggtaaaggcggtggaggatccggcggtggtggatcacaggtgcagctgcaggagtcggggggaggcctggtcaagcctggagggtccctgagactctcctgtgcagcctctggattcacctttagtagttattggatgagctgggtccgccaggctccagggaaggggctggagtgggtggccaacataaaccgcgatggaagtgcgagttactatgtggactctgtgaagggccgattcaccatctccagagacgacgccaagaactcactgtatctgcaaatgaacagcctgagagctgaggacacggctgtgtattactgtgcgagagatcgtggggtgggctacttcgatctctggggccgtggcaccctggtcaccgtctcgagcggtggaggcggttcaggcggaggtggttccggcggtggcggctcccagtctgccctgactcagcctgcctccgtgtctgggtctcctggacagtcgatcaccatctcctgcactggaaccagcagtgacgttggtggttataactttgtctcctggtaccaacaacacccaggcaaagcccccaaactcatgatctatgatgtcagtgatcggccctcaggggtgtctgatcgcttctccggctccaagtctggcaacacggcctccctgatcatctctggcctccaggctgacgacgaggctgattattactgcagctcatatgggagcagcagcactcatgtgattttcggcggagggaccaaggtgaccgtccta

SEQ ID NO: 64 - DNA, 357 bp, artificial sequence; identical to SEQ ID NO: 14
  Synthesized

SEQ ID NO: 65 - DNA, 732 bp, artificial sequence
  Synthesized
caggtgcagctgcaggagtcggggggaggcctggtcaagcctggagggtccctgagactctcctgtgcagcctctggattcacctttagtagttattggatgagctgggtccgccaggctccagggaaggggctggagtgggtggccaacataaaccgcgatggaagtgcgagttactatgtggactctgtgaagggccgattcaccatctccagagacgacgccaagaactcactgtatctgcaaatgaacagcctgagagctgaggacacggctgtgtattactgtgcgagagatcgtggggtgggctacttcgatctctggggccgtggcaccctggtcaccgtctcgagcggtggaggcggttcaggcggaggtggttccggcggtggcggctcccagtctgccctgactcagcctgcctccgtgtctgggtctcctggacagtcgatcaccatctcctgcactggaaccagcagtgacgttggtggttataactttgtctcctggtaccaacaacacccaggcaaagcccccaaactcatgatctatgatgtcagtgatcggccctcaggggtgtctgatcgcttctccggctccaagtctggcaacacggcctccctgatcatctctggcctccaggctgacgacgaggctgattattactgcagctcatatgggagcagcagcactcatgtgattttcggcggagggaccaaggtgaccgtccta

SEQ ID NO: 66 - protein, 703 aa, artificial sequence
  Synthesized
QVQLQESGPGLVKPSETLSLTCTVSGGSVSSGDYYWTWIRQSPGKGLEWIGHIYYSGNTNYNPSLKSRLTISIDTSKTQFSLKLSSVTAADTAIYYCVRDRVTGAFDIWGQGTMVTVSSASTKGPSVFPLAPSSKSTSGGTAALGCLVKDYFPEPVTVSWNSGALTSGVHTFPAVLQSSGLYSLSSVVTVPSSSLGTQTYICNVNHKPSNTKVDKRVEPKSCDKTHTCPPCPAPELLGGPSVFLFPPKPKDTLMISRTPEVTCVVVDVSHEDPEVKFNWYVDGVEVHNAKTKPREEQYNSTYRVVSVLTVLHQDWLNGKEYKCKVSNKALPAPIEKTISKAKGQPREPQVYTLPPSREEMTKNQVSLTCLVKGFYPSDIAVEWESNGQPENNYKTTPPVLDSDGSFFLYSKLTVDKSRWQQGNVFSCSVMHEALHNHYTQKSLSLSPGKGGGGSGGGGSQVQLQESGGGLVKPGGSLRLSCAASGFTFSSYWMSWVRQAPGKGLEWVANINRDGSASYYVDSVKGRFTISRDDAKNSLYLQMNSLRAEDTAVYYCARDRGVGYFDLWGRGTLVTVSSGGGGSGGGGSGGGGSQSALTQPASVSGSPGQSITISCTGTSSDVGGYNFVSWYQQHPGKAPKLMIYDVSDRPSGVSDRFSGSKSGNTASLIISGLQADDEADYYCSSYGSSSTHVIFGGGTKVTVL

SEQ ID NO: 67 - protein, 119 aa, artificial sequence [sequence omitted]

SEQ ID NO: 68 - protein, 243 aa, artificial sequence
  Synthesized
QVQLQESGGGLVKPGGSLRLSCAASGFTFSSYWMSWVRQAPGKGLEWVANINRDGSASYYVDSVKGRFTISRDDAKNSLYLQMNSLRAEDTAVYYCARDRGVGYFDLWGRGTLVTVSSGGGGSGGGGSGGGGSQSALTQPASVSGSPGQSITISCTGTSSDVGGYNFVSWYQQHPGKAPKLMIYDVSDRPSGVSDRFSGSKSGNTASLIISGLQADDEADYYCSSYGSSSTHVIFGGGTKVTV

SEQ ID NO: 69 - DNA, 654 bp, artificial sequence; identical to SEQ ID NO: 1
  Synthesized

SEQ ID NO: 70 - DNA, 333 bp, artificial sequence; identical to SEQ ID NO: 2
  Synthesized

SEQ ID NO: 71 - protein, 218 aa, artificial sequence; identical to SEQ ID NO: 3
  Synthesized

SEQ ID NO: 72 - protein, 111 aa, artificial sequence; identical to SEQ ID NO: 36
  Synthesized

SEQ ID NO: 73 - DNA, 2127 bp, artificial sequence
  Synthesized
caggtgcagctgcaggagtcggggggaggcctggtcaagcctggagggtccctgagactctcctgtgcagcctctggattcacctttagtagttattggatgagctgggtccgccaggctccagggaaggggctggagtgggtggccaacataaaccgcgatggaagtgcgagttactatgtggactctgtgaagggccgattcaccatctccagagacgacgccaagaactcactgtatctgcaaatgaacagcctgagagctgaggacacggctgtgtattactgtgcgagagatcgtggggtgggctacttcgatctctggggccgtggcaccctggtcaccgtctcgagcgctagcaccaagggcccatcggtcttccccctggcaccctcctccaagagcacctctgggggcacagcggccctgggctgcctggtcaaggactacttccccgaaccggtgacggtgtcgtggaactcaggcgccctgaccagcggcgtgcacaccttcccggctgtcctacagtcctcaggactctactccctcagcagcgtggtgaccgtgccctccagcagcttgggcacccagacctacatctgcaacgtgaatcacaagcccagcaacaccaaggtggacaagagagttgagcccaaatcttgtgacaaaactcacacatgcccaccgtgcccagcacctgaactcctggggggaccgtcagtcttcctcttccccccaaaacccaaggacaccctcatgatctcccggacccctgaggtcacatgcgtggtggtggacgtgagccacgaagaccctgaggtcaagttcaactggtacgtggacggcgtggaggtgcataatgccaagacaaagccgcgggaggagcagtacaacagcacgtaccgtgtggtcagcgtcctcaccgtcctgcaccaggactggctgaatggcaaggagtacaagtgcaaggtctccaacaaagccctcccagcccccatcgagaaaaccatctccaaagccaaagggcagccccgagaaccacaggtgtacaccctgcccccatcccgggaggagatgaccaagaaccaggtcagcctgacctgcctggtcaaaggcttctatcccagcgacatcgccgtggagtgggagagcaatgggcagccggagaacaactacaagaccacgcctcccgtgctggactccgacggctccttcttcctctatagcaagctcaccgtggacaagagcaggtggcagcaggggaacgtcttctcatgctccgtgatgcatgaggctctgcacaaccactacacgcagaagagcctctccctgtctccgggtaaaggcggtggaggatccggcggtggtggatcacaagttcaacttcaacaatctggtgctgaagttaaaaaacctggttcttctgttaaagtttcttgtaaagcctctggttatacttttactaattattatatttattgggttcgtcaagctcctggtcaaggtcttgaatggattggtggtattaatcctacttctggtggttctaattttaatgaaaaatttaaaactcgtgttactattactgttgatgaatctacgaacactgcttatatggaactttcttctcttcgttctgaagatactgctttttatttttgtgcgcgtcaaggtctttggtttgattctgatggtcgtggttttgatttttggggtcaaggttccactgttactgtctcgagcggtggaggcggttcaggcggaggtggttccggcggtggcggctccgatattcaaatgactcaatctccttcttctctttctgcttctgttggtgatcgtgttactattacttgtcgttcttctcaaaatattgttcattctaatggtaatacttatcttgattggtatcaacaaactcctggtaaagctcctaaacttcttatttataaagtttctaatcgtttttctggtgttccttctcgtttttctggttctggttctggtactgattttacttttactatttcttctcttcaacctgaagatattgctacttattattgttttcaatattctcatgttccttggacttttggtcaaggtactaaacttcaaattactcgt

SEQ ID NO: 74 - DNA, 354 bp, artificial sequence; identical to SEQ ID NO: 6
  Synthesized

SEQ ID NO: 75 - DNA, 753 bp, artificial sequence
  Synthesized
caagttcaacttcaacaatctggtgctgaagttaaaaaacctggttcttctgttaaagtttcttgtaaagcctctggttatacttttactaattattatatttattgggttcgtcaagctcctggtcaaggtcttgaatggattggtggtattaatcctacttctggtggttctaattttaatgaaaaatttaaaactcgtgttactattactgttgatgaatctacgaacactgcttatatggaactttcttctcttcgttctgaagatactgctttttatttttgtgcgcgtcaaggtctttggtttgattctgatggtcgtggttttgatttttggggtcaaggttccactgttactgtctcgagcggtggaggcggttcaggcggaggtggttccggcggtggcggctccgatattcaaatgactcaatctccttcttctctttctgcttctgttggtgatcgtgttactattacttgtcgttcttctcaaaatattgttcattctaatggtaatacttatcttgattggtatcaacaaactcctggtaaagctcctaaacttcttatttataaagtttctaatcgtttttctggtgttccttctcgtttttctggttctggttctggtactgattttacttttactatttcttctcttcaacctgaagatattgctacttattattgttttcaatattctcatgttccttggacttttggtcaaggtactaaacttcaaattactcgt

SEQ ID NO: 76 - protein, 709 aa, artificial sequence
  Synthesized
QVQLQESGGGLVKPGGSLRLSCAASGFTFSSYWMSWVRQAPGKGLEWVANINRDGSASYYVDSVKGRFTISRDDAKNSLYLQMNSLRAEDTAVYYCARDRGVGYFDLWGRGTLVTVSSASTKGPSVFPLAPSSKSTSGGTAALGCLVKDYFPEPVTVSWNSGALTSGVHTFPAVLQSSGLYSLSSVVTVPSSSLGTQTYICNVNHKPSNTKVDKRVEPKSCDKTHTCPPCPAPELLGGPSVFLFPPKPKDTLMISRTPEVTCVVVDVSHEDPEVKFNWYVDGVEVHNAKTKPREEQYNSTYRVVSVLTVLHQDWLNGKEYKCKVSNKALPAPIEKTISKAKGQPREPQVYTLPPSREEMTKNQVSLTCLVKGFYPSDIAVEWESNGQPENNYKTTPPVLDSDGSFFLYSKLTVDKSRWQQGNVFSCSVMHEALHNHYTQKSLSLSPGKGGGGSGGGGSQVQLQQSGAEVKKPGSSVKVSCKASGYTFTNYYIYWVRQAPGQGLEWIGGINPTSGGSNFNEKFKTRVTITVDESTNTAYMELSSLRSEDTAFYFCARQGLWFDSDGRGFDFWGQGSTVTVSSGGGGSGGGGSGGGGSDIQMTQSPSSLSASVGDRVTITCRSSQNIVHSNGNTYLDWYQQTPGKAPKLLIYKVSNRFSGVPSRFSGSGSGTDFTFTISSLQPEDIATYYCFQYSHVPWTFGQGTKLQITR

SEQ ID NO: 77 - protein, 118 aa, artificial sequence; identical to SEQ ID NO: 8
  Synthesized

SEQ ID NO: 78 - protein, 251 aa, artificial sequence
  Synthesized
QVQLQQSGAEVKKPGSSVKVSCKASGYTFTNYYIYWVRQAPGQGLEWIGGINPTSGGSNFNEKFKTRVTITVDESTNTAYMELSSLRSEDTAFYFCARQGLWFDSDGRGFDFWGQGSTVTVSSGGGGSGGGGSGGGGSDIQMTQSPSSLSASVGDRVTITCRSSQNIVHSNGNTYLDWYQQTPGKAPKLLIYKVSNRFSGVPSRFSGSGSGTDFTFTISSLQPEDIATYYCFQYSHVPWTFGQGTKLQITR

SEQ ID NO: 79 - DNA, 657 bp, artificial sequence; identical to SEQ ID NO: 25
  Synthesized

SEQ ID NO: 80 - DNA, 336 bp, artificial sequence; identical to SEQ ID NO: 26
  Synthesized

SEQ ID NO: 81 - protein, 219 aa, artificial sequence; identical to SEQ ID NO: 27
  Synthesized

SEQ ID NO: 82 - protein, 112 aa, artificial sequence [sequence omitted]

SEQ ID NO: 83 - DNA, 2121 bp, artificial sequence
  Synthesized
caagttcaacttcaacaatctggtgctgaagttaaaaaacctggttcttctgttaaagtttcttgtaaagcctctggttatacttttactaattattatatttattgggttcgtcaagctcctggtcaaggtcttgaatggattggtggtattaatcctacttctggtggttctaattttaatgaaaaatttaaaactcgtgttactattactgttgatgaatctacgaacactgcttatatggaactttcttctcttcgttctgaagatactgctttttatttttgtgcgcgtcaaggtctttggtttgattctgatggtcgtggttttgatttttggggtcaaggttccactgttactgtctcgagcgctagcaccaagggcccatcggtcttccccctggcaccctcctccaagagcacctctgggggcacagcggccctgggctgcctggtcaaggactacttccccgaaccggtgacggtgtcgtggaactcaggcgccctgaccagcggcgtgcacaccttcccggctgtcctacagtcctcaggactctactccctcagcagcgtggtgaccgtgccctccagcagcttgggcacccagacctacatctgcaacgtgaatcacaagcccagcaacaccaaggtggacaagagagttgagcccaaatcttgtgacaaaactcacacatgcccaccgtgcccagcacctgaactcctggggggaccgtcagtcttcctcttccccccaaaacccaaggacaccctcatgatctcccggacccctgaggtcacatgcgtggtggtggacgtgagccacgaagaccctgaggtcaagttcaactggtacgtggacggcgtggaggtgcataatgccaagacaaagccgcgggaggagcagtacaacagcacgtaccgtgtggtcagcgtcctcaccgtcctgcaccaggactggctgaatggcaaggagtacaagtgcaaggtctccaacaaagccctcccagcccccatcgagaaaaccatctccaaagccaaagggcagccccgagaaccacaggtgtacaccctgcccccatcccgggaggagatgaccaagaaccaggtcagcctgacctgcctggtcaaaggcttctatcccagcgacatcgccgtggagtgggagagcaatgggcagccggagaacaactacaagaccacgcctcccgtgctggactccgacggctccttcttcctctatagcaagctcaccgtggacaagagcaggtggcagcaggggaacgtcttctcatgctccgtgatgcatgaggctctgcacaaccactacacgcagaagagcctctccctgtctccgggtaaaggcggtggaggatccggcggtggtggatcacaggtgcagctgcaggagtcggggggaggcctggtcaagcctggagggtccctgagactctcctgtgcagcctctggattcacctttagtagttattggatgagctgggtccgccaggctccagggaaggggctggagtgggtggccaacataaaccgcgatggaagtgcgagttactatgtggactctgtgaagggccgattcaccatctccagagacgacgccaagaactcactgtatctgcaaatgaacagcctgagagctgaggacacggctgtgtattactgtgcgagagatcgtggggtgggctacttcgatctctggggccgtggcaccctggtcaccgtctcgagcggtggaggcggttcaggcggaggtggttccggcggtggcggctcccagtctgccctgactcagcctgcctccgtgtctgggtctcctggacagtcgatcaccatctcctgcactggaaccagcagtgacgttggtggttataactttgtctcctggtaccaacaacacccaggcaaagcccccaaactcatgatctatgatgtcagtgatcggccctcaggggtgtctgatcgcttctccggctccaagtctggcaacacggcctccctgatcatctctggcctccaggctgacgacgaggctgattattactgcagctcatatgggagcagcagcactcatgtgattttcggcggagggaccaaggtgaccgtccta

SEQ ID NO: 84 - DNA, 369 bp, artificial sequence; identical to SEQ ID NO: 30
  Synthesized

SEQ ID NO: 85 - DNA, 732 bp, artificial sequence; identical to SEQ ID NO: 65
  Synthesized

SEQ ID NO: 86 - protein, 707 aa, artificial sequence
  Synthesized
QVQLQQSGAEVKKPGSSVKVSCKASGYTFTNYYIYWVRQAPGQGLEWIGGINPTSGGSNFNEKFKTRVTITVDESTNTAYMELSSLRSEDTAFYFCARQGLWFDSDGRGFDFWGQGSTVTVSSASTKGPSVFPLAPSSKSTSGGTAALGCLVKDYFPEPVTVSWNSGALTSGVHTFPAVLQSSGLYSLSSVVTVPSSSLGTQTYICNVNHKPSNTKVDKRVEPKSCDKTHTCPPCPAPELLGGPSVFLFPPKPKDTLMISRTPEVTCVVVDVSHEDPEVKFNWYVDGVEVHNAKTKPREEQYNSTYRVVSVLTVLHQDWLNGKEYKCKVSNKALPAPIEKTISKAKGQPREPQVYTLPPSREEMTKNQVSLTCLVKGFYPSDIAVEWESNGQPENNYKTTPPVLDSDGSFFLYSKLTVDKSRWQQGNVFSCSVMHEALHNHYTQKSLSLSPGKGGGGSGGGGSQVQLQESGGGLVKPGGSLRLSCAASGFTFSSYWMSWVRQAPGKGLEWVANINRDGSASYYVDSVKGRFTISRDDAKNSLYLQMNSLRAEDTAVYYCARDRGVGYFDLWGRGTLVTVSSGGGGSGGGGSGGGGSQSALTQPASVSGSPGQSITISCTGTSSDVGGYNFVSWYQQHPGKAPKLMIYDVSDRPSGVSDRFSGSKSGNTASLIISGLQADDEADYYCSSYGSSSTHVIFGGGTKVTVL

SEQ ID NO: 87 - protein, 123 aa, artificial sequence; identical to SEQ ID NO: 32
  Synthesized

SEQ ID NO: 88 - protein, 244 aa, artificial sequence
  Synthesized
QVQLQESGGGLVKPGGSLRLSCAASGFTFSSYWMSWVRQAPGKGLEWVANINRDGSASYYVDSVKGRFTISRDDAKNSLYLQMNSLRAEDTAVYYCARDRGVGYFDLWGRGTLVTVSSGGGGSGGGGSGGGGSQSALTQPASVSGSPGQSITISCTGTSSDVGGYNFVSWYQQHPGKAPKLMIYDVSDRPSGVSDRFSGSKSGNTASLIISGLQADDEADYYCSSYGSSSTHVIFGGGTKVTVL

SEQ ID NO: 89 - DNA, 657 bp, artificial sequence; identical to SEQ ID NO: 25
  Synthesized

SEQ ID NO: 90 - DNA, 336 bp, artificial sequence; identical to SEQ ID NO: 26
  Synthesized

SEQ ID NO: 91 - DNA, 336 bp, artificial sequence
  Synthesized
gacatccagatgacccagtccccttccagcctgtccgcttccgtgggcgacagggtgaccatcacctgcaggtcctcccagaacatcgtgcactccaacggcaatacctacctggactggtaccagcagacccccggcaaggcccctaagctgctgatctacaaggtgagcaaccggttcagcggcgtgccttcccggttttccggatccggctccggcacagacttcaccttcaccatctcctccctgcaacccgaggacatcgccacctactactgcttccagtactcccatgtgccctggaccttcggccagggcaccaagctgcagatcacc

SEQ ID NO: 92 - protein, 218 aa, artificial sequence; identical to SEQ ID NO: 3
  Synthesized

SEQ ID NO: 93 - protein, 111 aa, artificial sequence; identical to SEQ ID NO: 36
  Synthesized

SEQ ID NO: 94 - DNA, 2118 bp, artificial sequence
  Synthesized
caggtgcagctgcagcagagcggcgccgaggtgaagaagcccggcagcagcgtgaaggtgagctgcaaggccagcggctacaccttcaccaactactacatctactgggtgcggcaggcccccggccagggcctggagtggatcggcggcatcaaccccaccagcggcggcagcaacttcaacgagaagttcaagacccgggtgaccatcaccgccgacgagagcagcaccaccgcctacatggagctgagcagcctgcggagcgaggacaccgccttctacttctgcacccggcagggcctgtggttcgacagcgacggccggggcttcgacttctggggccagggcaccaccgtgaccgtgagcagcgctagcaccaagggcccatcggtcttccccctggcaccctcctccaagagcacctctgggggcacagcggccctgggctgcctggtcaaggactacttccccgaaccggtgacggtgtcgtggaactcaggcgccctgaccagcggcgtgcacaccttcccggctgtcctacagtcctcaggactctactccctcagcagcgtggtgaccgtgccctccagcagcttgggcacccagacctacatctgcaacgtgaatcacaagcccagcaacaccaaggtggacaagagagttgagcccaaatcttgtgacaaaactcacacatgcccaccgtgcccagcacctgaactcctggggggaccgtcagtcttcctcttccccccaaaacccaaggacaccctcatgatctcccggacccctgaggtcacatgcgtggtggtggacgtgagccacgaagaccctgaggtcaagttcaactggtacgtggacggcgtggaggtgcataatgccaagacaaagccgcgggaggagcagtacaacagcacgtaccgtgtggtcagcgtcctcaccgtcctgcaccaggactggctgaatggcaaggagtacaagtgcaaggtctccaacaaagccctcccagcccccatcgagaaaaccatctccaaagccaaagggcagccccgagaaccacaggtgtacaccctgcccccatcccgggatgagctgaccaagaaccaggtcagcctgacctgcctggtcaaaggcttctatcccagcgacatcgccgtggagtgggagagcaatgggcagccggagaacaactacaagaccacgcctcccgtgctggactccgacggctccttcttcctctatagcaagctcaccgtggacaagagcaggtggcagcaggggaacgtcttctcatgctccgtgatgcatgaggctctgcacaaccactacacgcagaagagcctctccctgtctccgggtggcggtggagggtccggcggtggtggatcacaggtgcaattgcaggagtcggggggaggcctggtcaagcctggagggtccctgagactctcctgtgcagcctctggattcacctttagtagttattggatgagctgggtccgccaggctccagggaaggggctggagtgggtggccaacataaaccgcgatggaagtgcgagttactatgtggactctgtgaagggccgattcaccatctccagagacgacgccaagaactcactgtatctgcaaatgaacagcctgagagctgaggacacggctgtgtattactgtgcgagagatcgtggggtgggctacttcgatctctggggccgtggcaccctggtcaccgtctcgagcggtggaggcggttcaggcggaggtggttccggcggtggcggctcccagtctgccctgactcagcctgcctccgtgtctgggtctcctggacagtcgatcaccatctcctgcactggaaccagcagtgacgttggtggttataactttgtctcctggtaccaacaacacccaggcaaagcccccaaactcatgatctatgatgtcagtgatcggccctcaggggtgtctgatcgcttctccggctccaagtctggcaacacggcctccctgatcatctctggcctccaggctgacgacgaggctgattattactgcagctcatatgggagcagcagcactcatgtgattttcggcggagggaccaaggtgaccgtccta

SEQ ID NO: 95 - DNA, 369 bp, artificial sequence; identical to SEQ ID NO: 38
  Synthesized

SEQ ID NO: 96 - DNA, 369 bp, artificial sequence
  Synthesized
caggtgcagctgcagcaatccggcgccgaggtgaagaagcctggctccagcgtgaaggtgtcctgcaaggcctccggctacaccttcaccaactactacatctactgggtgaggcaggctcctggccagggactggagtggatcggcggcatcaaccctacctccggcggctccaacttcaacgagaagttcaagacccgggtgaccatcaccgccgatgagagctccaccaccgcctacatggagctgtcctccctgaggtccgaggacaccgccttttacttctgcaccaggcagggactgtggttcgactccgacggccggggcttcgatttttggggccagggcaccacagtgaccgtgtcctcc

SEQ ID NO: 97 - DNA, 732 bp, artificial sequence
  Synthesized
caggtgcaattgcaggagtcggggggaggcctggtcaagcctggagggtccctgagactctcctgtgcagcctctggattcacctttagtagttattggatgagctgggtccgccaggctccagggaaggggctggagtgggtggccaacataaaccgcgatggaagtgcgagttactatgtggactctgtgaagggccgattcaccatctccagagacgacgccaagaactcactgtatctgcaaatgaacagcctgagagctgaggacacggctgtgtattactgtgcgagagatcgtggggtgggctacttcgatctctggggccgtggcaccctggtcaccgtctcgagcggtggaggcggttcaggcggaggtggttccggcggtggcggctcccagtctgccctgactcagcctgcctccgtgtctgggtctcctggacagtcgatcaccatctcctgcactggaaccagcagtgacgttggtggttataactttgtctcctggtaccaacaacacccaggcaaagcccccaaactcatgatctatgatgtcagtgatcggccctcaggggtgtctgatcgcttctccggctccaagtctggcaacacggcctccctgatcatctctggcctccaggctgacgacgaggctgattattactgcagctcatatgggagcagcagcactcatgtgattttcggcggagggaccaaggtgaccgtccta

SEQ ID NO: 98 - protein, 706 aa, artificial sequence
  Synthesized
QVQLQQSGAEVKKPGSSVKVSCKASGYTFTNYYIYWVRQAPGQGLEWIGGINPTSGGSNFNEKFKTRVTITADESSTTAYMELSSLRSEDTAFYFCTRQGLWFDSDGRGFDFWGQGTTVTVSSASTKGPSVFPLAPSSKSTSGGTAALGCLVKDYFPEPVTVSWNSGALTSGVHTFPAVLQSSGLYSLSSVVTVPSSSLGTQTYICNVNHKPSNTKVDKRVEPKSCDKTHTCPPCPAPELLGGPSVFLFPPKPKDTLMISRTPEVTCVVVDVSHEDPEVKFNWYVDGVEVHNAKTKPREEQYNSTYRVVSVLTVLHQDWLNGKEYKCKVSNKALPAPIEKTISKAKGQPREPQVYTLPPSRDELTKNQVSLTCLVKGFYPSDIAVEWESNGQPENNYKTTPPVLDSDGSFFLYSKLTVDKSRWQQGNVFSCSVMHEALHNHYTQKSLSLSPGGGGGSGGGGSQVQLQESGGGLVKPGGSLRLSCAASGFTFSSYWMSWVRQAPGKGLEWVANINRDGSASYYVDSVKGRFTISRDDAKNSLYLQMNSLRAEDTAVYYCARDRGVGYFDLWGRGTLVTVSSGGGGSGGGGSGGGGSQSALTQPASVSGSPGQSITISCTGTSSDVGGYNFVSWYQQHPGKAPKLMIYDVSDRPSGVSDRFSGSKSGNTASLIISGLQADDEADYYCSSYGSSSTHVIFGGGTKVTVL

SEQ ID NO: 99 - protein, 123 aa, artificial sequence [sequence omitted]

SEQ ID NO: 100 - protein, 244 aa, artificial sequence; identical to SEQ ID NO: 88
  Synthesized

SEQ ID NO: 101 - DNA, 654 bp, artificial sequence; identical to SEQ ID NO: 1
  Synthesized

SEQ ID NO: 102 - DNA, 333 bp, artificial sequence; identical to SEQ ID NO: 2
  Synthesized

SEQ ID NO: 103 - protein, 218 aa, artificial sequence; identical to SEQ ID NO: 3
  Synthesized

SEQ ID NO: 104 - protein, 111 aa, artificial sequence; identical to SEQ ID NO: 36
  Synthesized

SEQ ID NO: 105 - DNA, 2100 bp, artificial sequence
  Synthesized
caggtgcagctgcaggagtcggggggaggcctggtcaagcctggagggtccctgagactctcctgtgcagcctctggattcacctttagtagttattggatgagctgggtccgccaggctccagggaaggggctggagtgggtggccaacataaaccgcgatggaagtgcgagttactatgtggactctgtgaagggccgattcaccatctccagagacgacgccaagaactcactgtatctgcaaatgaacagcctgagagctgaggacacggctgtgtattactgtgcgagagatcgtggggtgggctacttcgatctctggggccgtggcaccctggtcaccgtctcgagcgctagcaccaagggcccatcggtcttccccctggcaccctcctccaagagcacctctgggggcacagcggccctgggctgcctggtcaaggactacttccccgaaccggtgacggtgtcgtggaactcaggcgccctgaccagcggcgtgcacaccttcccggctgtcctacagtcctcaggactctactccctcagcagcgtggtgaccgtgccctccagcagcttgggcacccagacctacatctgcaacgtgaatcacaagcccagcaacaccaaggtggacaagagagttgagcccaaatcttgtgacaaaactcacacatgcccaccgtgcccagcacctgaactcctggggggaccgtcagtcttcctcttccccccaaaacccaaggacaccctcatgatctcccggacccctgaggtcacatgcgtggtggtggacgtgagccacgaagaccctgaggtcaagttcaactggtacgtggacggcgtggaggtgcataatgccaagacaaagccgcgggaggagcagtacaacagcacgtaccgtgtggtcagcgtcctcaccgtcctgcaccaggactggctgaatggcaaggagtacaagtgcaaggtctccaacaaagccctcccagcccccatcgagaaaaccatctccaaagccaaagggcagccccgagaaccacaggtgtacaccctgcccccatcccgggaggagatgaccaagaaccaggtcagcctgacctgcctggtcaaaggcttctatcccagcgacatcgccgtggagtgggagagcaatgggcagccggagaacaactacaagaccacgcctcccgtgctggactccgacggctccttcttcctctatagcaagctcaccgtggacaagagcaggtggcagcaggggaacgtcttctcatgctccgtgatgcatgaggctctgcacaaccactacacgcagaagagcctctccctgtctccgggtaaaggcggtggaggatccggcggtggtggatcacaggtgcagctgaagcagtcaggacctggcctagtgcagccctcacagagcctgtccatcacctgcacagtctctggtttctcattaactaactatggtgtacactgggttcgccagtctccaggaaagggtctggagtggctgggagtgatatggagtggtggaaacacagactataatacacctttcacatccagactgagcatcaacaaggacaattccaagagccaagttttctttaaaatgaacagtctgcaatctaatgacacagccatatattactgtgccagagccctcacctactatgattacgagtttgcttactggggccaagggactctggtcactgtctctagcggtggaggcggttcaggcggaggtggttccggcggtggcggctccgacatcttgctgactcagtctccagtcatcctgtctgtgagtccaggagaaagagtcagtttctcctgcagggccagtcagagtattggcacaaacatacactggtatcagcaaagaacaaatggttctccaaggcttctcataaagtatgcttctgagtctatctctgggattccttccaggtttagtggcagtggatcagggacagattttactcttagcatcaacagtgtggagtctgaagatattgcagattattactgtcaacaaaataataactggccaaccacgttcggtgctgggaccaagctggagctgaaacgt

SEQ ID NO: 106 - DNA, 354 bp, artificial sequence; identical to SEQ ID NO: 6
  Synthesized

SEQ ID NO: 107 - DNA, 726 bp, artificial sequence
  Synthesized
caggtgcagctgaagcagtcaggacctggcctagtgcagccctcacagagcctgtccatcacctgcacagtctctggtttctcattaactaactatggtgtacactgggttcgccagtctccaggaaagggtctggagtggctgggagtgatatggagtggtggaaacacagactataatacacctttcacatccagactgagcatcaacaaggacaattccaagagccaagttttctttaaaatgaacagtctgcaatctaatgacacagccatatattactgtgccagagccctcacctactatgattacgagtttgcttactggggccaagggactctggtcactgtctctagcggtggaggcggttcaggcggaggtggttccggcggtggcggctccgacatcttgctgactcagtctccagtcatcctgtctgtgagtccaggagaaagagtcagtttctcctgcagggccagtcagagtattggcacaaacatacactggtatcagcaaagaacaaatggttctccaaggcttctcataaagtatgcttctgagtctatctctgggattccttccaggtttagtggcagtggatcagggacagattttactcttagcatcaacagtgtggagtctgaagatattgcagattattactgtcaacaaaataataactggccaaccacgttcggtgctgggaccaagctggagctgaaacgt

SEQ ID NO: 108 - protein, 700 aa, artificial sequence
  Synthesized
QVQLQESGGGLVKPGGSLRLSCAASGFTFSSYWMSWVRQAPGKGLEWVANINRDGSASYYVDSVKGRFTISRDDAKNSLYLQMNSLRAEDTAVYYCARDRGVGYFDLWGRGTLVTVSSASTKGPSVFPLAPSSKSTSGGTAALGCLVKDYFPEPVTVSWNSGALTSGVHTFPAVLQSSGLYSLSSVVTVPSSSLGTQTYICNVNHKPSNTKVDKRVEPKSCDKTHTCPPCPAPELLGGPSVFLFPPKPKDTLMISRTPEVTCVVVDVSHEDPEVKFNWYVDGVEVHNAKTKPREEQYNSTYRVVSVLTVLHQDWLNGKEYKCKVSNKALPAPIEKTISKAKGQPREPQVYTLPPSREEMTKNQVSLTCLVKGFYPSDIAVEWESNGQPENNYKTTPPVLDSDGSFFLYSKLTVDKSRWQQGNVFSCSVMHEALHNHYTQKSLSLSPGKGGGGSGGGGSQVQLKQSGPGLVQPSQSLSITCTVSGFSLTNYGVHWVRQSPGKGLEWLGVIWSGGNTDYNTPFTSRLSINKDNSKSQVFFKMNSLQSNDTAIYYCARALTYYDYEFAYWGQGTLVTVSSGGGGSGGGGSGGGGSDILLTQSPVILSVSPGERVSFSCRASQSIGTNIHWYQQRTNGSPRLLIKYASESISGIPSRFSGSGSGTDFTLSINSVESEDIADYYCQQNNNWPTTFGAGTKLELKR

SEQ ID NO: 109 - protein, 118 aa, artificial sequence; identical to SEQ ID NO: 8
  Synthesized

SEQ ID NO: 110 - protein, 242 aa, artificial sequence
  Synthesized
QVQLKQSGPGLVQPSQSLSITCTVSGFSLTNYGVHWVRQSPGKGLEWLGVIWSGGNTDYNTPFTSRLSINKDNSKSQVFFKMNSLQSNDTAIYYCARALTYYDYEFAYWGQGTLVTVSSGGGGSGGGGSGGGGSDILLTQSPVILSVSPGERVSFSCRASQSIGTNIHWYQQRTNGSPRLLIKYASESISGIPSRFSGSGSGTDFTLSINSVESEDIADYYCQQNNNWPTTFGAGTKLELKR

SEQ ID NO: 111 - DNA, 642 bp, artificial sequence; identical to SEQ ID NO: 41
  Synthesized

SEQ ID NO: 112 - DNA, 321 bp, artificial sequence; identical to SEQ ID NO: 42
  Synthesized

SEQ ID NO: 113 - protein, 214 aa, artificial sequence; identical to SEQ ID NO: 43
  Synthesized

SEQ ID NO: 114 - protein, 107 aa, artificial sequence; identical to SEQ ID NO: 44
  Synthesized

SEQ ID NO: 115 - DNA, 2109 bp, artificial sequence
  Synthesized
caggtgcagctgaagcagtcaggacctggcctagtgcagccctcacagagcctgtccatcacctgcacagtctctggtttctcattaactaactatggtgtacactgggttcgccagtctccaggaaagggtctggagtggctgggagtgatatggagtggtggaaacacagactataatacacctttcacatccagactgagcatcaacaaggacaattccaagagccaagttttctttaaaatgaacagtctgcaatctaatgacacagccatatattactgtgccagagccctcacctactatgattacgagtttgcttactggggccaagggactctggtcactgtctctagcgctagcaccaagggcccatcggtcttccccctggcaccctcctccaagagcacctctgggggcacagcggccctgggctgcctggtcaaggactacttccccgaaccggtgacggtgtcgtggaactcaggcgccctgaccagcggcgtgcacaccttcccggctgtcctacagtcctcaggactctactccctcagcagcgtggtgaccgtgccctccagcagcttgggcacccagacctacatctgcaacgtgaatcacaagcccagcaacaccaaggtggacaagagagttgagcccaaatcttgtgacaaaactcacacatgcccaccgtgcccagcacctgaactcctggggggaccgtcagtcttcctcttccccccaaaacccaaggacaccctcatgatctcccggacccctgaggtcacatgcgtggtggtggacgtgagccacgaagaccctgaggtcaagttcaactggtacgtggacggcgtggaggtgcataatgccaagacaaagccgcgggaggagcagtacaacagcacgtaccgtgtggtcagcgtcctcaccgtcctgcaccaggactggctgaatggcaaggagtacaagtgcaaggtctccaacaaagccctcccagcccccatcgagaaaaccatctccaaagccaaagggcagccccgagaaccacaggtgtacaccctgcccccatcccgggaggagatgaccaagaaccaggtcagcctgacctgcctggtcaaaggcttctatcccagcgacatcgccgtggagtgggagagcaatgggcagccggagaacaactacaagaccacgcctcccgtgctggactccgacggctccttcttcctctatagcaagctcaccgtggacaagagcaggtggcagcaggggaacgtcttctcatgctccgtgatgcatgaggctctgcacaaccactacacgcagaagagcctctccctgtctccgggtaaaggcggtggaggatccggcggtggtggatcacaggtgcagctgcaggagtcggggggaggcctggtcaagcctggagggtccctgagactctcctgtgcagcctctggattcacctttagtagttattggatgagctgggtccgccaggctccagggaaggggctggagtgggtggccaacataaaccgcgatggaagtgcgagttactatgtggactctgtgaagggccgattcaccatctccagagacgacgccaagaactcactgtatctgcaaatgaacagcctgagagctgaggacacggctgtgtattactgtgcgagagatcgtggggtgggctacttcgatctctggggccgtggcaccctggtcaccgtctcgagcggtggaggcggttcaggcggaggtggttccggcggtggcggctcccagtctgccctgactcagcctgcctccgtgtctgggtctcctggacagtcgatcaccatctcctgcactggaaccagcagtgacgttggtggttataactttgtctcctggtaccaacaacacccaggcaaagcccccaaactcatgatctatgatgtcagtgatcggccctcaggggtgtctgatcgcttctccggctccaagtctggcaacacggcctccctgatcatctctggcctccaggctgacgacgaggctgattattactgcagctcatatgggagcagcagcactcatgtgattttcggcggagggaccaaggtgaccgtccta

SEQ ID NO: 116 - DNA, 357 bp, artificial sequence; identical to SEQ ID NO: 46
  Synthesized

SEQ ID NO: 117 - DNA, 732 bp, artificial sequence; identical to SEQ ID NO: 65
  Synthesized

SEQ ID NO: 118 - protein, 703 aa, artificial sequence
  Synthesized
QVQLKQSGPGLVQPSQSLSITCTVSGFSLTNYGVHWVRQSPGKGLEWLGVIWSGGNTDYNTPFTSRLSINKDNSKSQVFFKMNSLQSNDTAIYYCARALTYYDYEFAYWGQGTLVTVSSASTKGPSVFPLAPSSKSTSGGTAALGCLVKDYFPEPVTVSWNSGALTSGVHTFPAVLQSSGLYSLSSVVTVPSSSLGTQTYICNVNHKPSNTKVDKRVEPKSCDKTHTCPPCPAPELLGGPSVFLFPPKPKDTLMISRTPEVTCVVVDVSHEDPEVKFNWYVDGVEVHNAKTKPREEQYNSTYRVVSVLTVLHQDWLNGKEYKCKVSNKALPAPIEKTISKAKGQPREPQVYTLPPSREEMTKNQVSLTCLVKGFYPSDIAVEWESNGQPENNYKTTPPVLDSDGSFFLYSKLTVDKSRWQQGNVFSCSVMHEALHNHYTQKSLSLSPGKGGGGSGGGGSQVQLQESGGGLVKPGGSLRLSCAASGFTFSSYWMSWVRQAPGKGLEWVANINRDGSASYYVDSVKGRFTISRDDAKNSLYLQMNSLRAEDTAVYYCARDRGVGYFDLWGRGTLVTVSSGGGGSGGGGSGGGGSQSALTQPASVSGSPGQSITISCTGTSSDVGGYNFVSWYQQHPGKAPKLMIYDVSDRPSGVSDRFSGSKSGNTASLIISGLQADDEADYYCSSYGSSSTHVIFGGGTKVTVL

SEQ ID NO: 119 - protein, 119 aa, artificial sequence; identical to SEQ ID NO: 48
  Synthesized

SEQ ID NO: 120 - protein, 244 aa, artificial sequence; identical to SEQ ID NO: 88
  Synthesized

SEQ ID NO: 121 - DNA, 642 bp, artificial sequence; identical to SEQ ID NO: 41
  Synthesized

SEQ ID NO: 122 - DNA, 321 bp, artificial sequence; identical to SEQ ID NO: 42
  Synthesized

SEQ ID NO: 123 - protein, 214 aa, artificial sequence; identical to SEQ ID NO: 43
  Synthesized

SEQ ID NO: 124 - protein, 107 aa, artificial sequence; identical to SEQ ID NO: 44
  Synthesized

SEQ ID NO: 125 - DNA, 1344 bp, artificial sequence
  Synthesized
caggtgcagctgaagcagtcaggacctggcctagtgcagccctcacagagcctgtccatcacctgcacagtctctggtttctcattaactaactatggtgtacactgggttcgccagtctccaggaaagggtctggagtggctgggagtgatatggagtggtggaaacacagactataatacacctttcacatccagactgagcatcaacaaggacaattccaagagccaagttttctttaaaatgaacagtctgcaatctaatgacacagccatatattactgtgccagagccctcacctactatgattacgagtttgcttactggggccaagggactctggtcactgtctctagcgctagcaccaagggcccatcggtcttccccctggcaccctcctccaagagcacctctgggggcacagcggccctgggctgcctggtcaaggactacttccccgaaccggtgacggtgtcgtggaactcaggcgccctgaccagcggcgtgcacaccttcccggctgtcctacagtcctcaggactctactccctcagcagcgtggtgaccgtgccctccagcagcttgggcacccagacctacatctgcaacgtgaatcacaagcccagcaacaccaaggtggacaagagagttgagcccaaatcttgtgacaaaactcacacatgcccaccgtgcccagcacctgaactcctggggggaccgtcagtcttcctcttccccccaaaacccaaggacaccctcatgatctcccggacccctgaggtcacatgcgtggtggtggacgtgagccacgaagaccctgaggtcaagttcaactggtacgtggacggcgtggaggtgcataatgccaagacaaagccgcgggaggagcagtacaacagcacgtaccgtgtggtcagcgtcctcaccgtcctgcaccaggactggctgaatggcaaggagtacaagtgcaaggtctccaacaaagccctcccagcccccatcgagaaaaccatctccaaagccaaagggcagccccgagaaccacaggtgtacaccctgcccccatcccgggatgagctgaccaagaaccaggtcagcctgacctgcctggtcaaaggcttctatcccagcgacatcgccgtggagtgggagagcaatgggcagccggagaacaactacaagaccacgcctcccgtgctggactccgacggctccttcttcctctatagcaagctcaccgtggacaagagcaggtggcagcaggggaacgtcttctcatgctccgtgatgcatgaggctctgcacaaccactacacgcagaagagcctctccctgtctccgggt

SEQ ID NO: 126 - DNA, 357 bp, artificial sequence; identical to SEQ ID NO: 46
  Synthesized

SEQ ID NO: 127 - protein, 448 aa, artificial sequence
  Synthesized
QVQLKQSGPGLVQPSQSLSITCTVSGFSLTNYGVHWVRQSPGKGLEWLGVIWSGGNTDYNTPFTSRLSINKDNSKSQVFFKMNSLQSNDTAIYYCARALTYYDYEFAYWGQGTLVTVSSASTKGPSVFPLAPSSKSTSGGTAALGCLVKDYFPEPVTVSWNSGALTSGVHTFPAVLQSSGLYSLSSVVTVPSSSLGTQTYICNVNHKPSNTKVDKRVEPKSCDKTHTCPPCPAPELLGGPSVFLFPPKPKDTLMISRTPEVTCVVVDVSHEDPEVKFNWYVDGVEVHNAKTKPREEQYNSTYRVVSVLTVLHQDWLNGKEYKCKVSNKALPAPIEKTISKAKGQPREPQVYTLPPSRDELTKNQVSLTCLVKGFYPSDIAVEWESNGQPENNYKTTPPVLDSDGSFFLYSKLTVDKSRWQQGNVFSCSVMHEALHNHYTQKSLSLSPG

SEQ ID NO: 128 - protein, 119 aa, artificial sequence; identical to SEQ ID NO: 48
  Synthesized

SEQ ID NO: 129 - DNA, 642 bp, artificial sequence; identical to SEQ ID NO: 41
  Synthesized

SEQ ID NO: 130 - DNA, 321 bp, artificial sequence; identical to SEQ ID NO: 42
  Synthesized

SEQ ID NO: 131 - protein, 214 aa, artificial sequence; identical to SEQ ID NO: 43
  Synthesized

SEQ ID NO: 132 - protein, 107 aa, artificial sequence; identical to SEQ ID NO: 44
  Synthesized

SEQ ID NO: 133 - DNA, 2106 bp, artificial sequence
  Synthesized
caggtgcagctgaagcagtcaggacctggcctagtgcagccctcacagagcctgtccatcacctgcacagtctctggtttctcattaactaactatggtgtacactgggttcgccagtctccaggaaagggtctggagtggctgggagtgatatggagtggtggaaacacagactataatacacctttcacatccagactgagcatcaacaaggacaattccaagagccaagttttctttaaaatgaacagtctgcaatctaatgacacagccatatattactgtgccagagccctcacctactatgattacgagtttgcttactggggccaagggactctggtcactgtctctagcgctagcaccaagggcccatcggtcttccccctggcaccctcctccaagagcacctctgggggcacagcggccctgggctgcctggtcaaggactacttccccgaaccggtgacggtgtcgtggaactcaggcgccctgaccagcggcgtgcacaccttcccggctgtcctacagtcctcaggactctactccctcagcagcgtggtgaccgtgccctccagcagcttgggcacccagacctacatctgcaacgtgaatcacaagcccagcaacaccaaggtggacaagagagttgagcccaaatcttgtgacaaaactcacacatgcccaccgtgcccagcacctgaactcctggggggaccgtcagtcttcctcttccccccaaaacccaaggacaccctcatgatctcccggacccctgaggtcacatgcgtggtggtggacgtgagccacgaagaccctgaggtcaagttcaactggtacgtggacggcgtggaggtgcataatgccaagacaaagccgcgggaggagcagtacaacagcacgtaccgtgtggtcagcgtcctcaccgtcctgcaccaggactggctgaatggcaaggagtacaagtgcaaggtctccaacaaagccctcccagcccccatcgagaaaaccatctccaaagccaaagggcagccccgagaaccacaggtgtacaccctgcccccatcccgggatgagctgaccaagaaccaggtcagcctgacctgcctggtcaaaggcttctatcccagcgacatcgccgtggagtgggagagcaatgggcagccggagaacaactacaagaccacgcctcccgtgctggactccgacggctccttcttcctctatagcaagctcaccgtggacaagagcaggtggcagcaggggaacgtcttctcatgctccgtgatgcatgaggctctgcacaaccactacacgcagaagagcctctccctgtctccgggtggcggtggagggtccggcggtggtggatcacaggtgcaattgcaggagtcggggggaggcctggtcaagcctggagggtccctgagactctcctgtgcagcctctggattcacctttagtagttattggatgagctgggtccgccaggctccagggaaggggctggagtgggtggccaacataaaccgcgatggaagtgcgagttactatgtggactctgtgaagggccgattcaccatctccagagacgacgccaagaactcactgtatctgcaaatgaacagcctgagagctgaggacacggctgtgtattactgtgcgagagatcgtggggtgggctacttcgatctctggggccgtggcaccctggtcaccgtctcgagcggtggaggcggttcaggcggaggtggttccggcggtggcggctcccagtctgccctgactcagcctgcctccgtgtctgggtctcctggacagtcgatcaccatctcctgcactggaaccagcagtgacgttggtggttataactttgtctcctggtaccaacaacacccaggcaaagcccccaaactcatgatctatgatgtcagtgatcggccctcaggggtgtctgatcgcttctccggctccaagtctggcaacacggcctccctgatcatctctggcctccaggctgacgacgaggctgattattactgcagctcatatgggagcagcagcactcatgtgattttcggcggagggaccaaggtgaccgtccta

SEQ ID NO: 134 - DNA, 357 bp, artificial sequence; identical to SEQ ID NO: 46
  Synthesized

SEQ ID NO: 135 - DNA, 732 bp, artificial sequence; identical to SEQ ID NO: 65
  Synthesized

SEQ ID NO: 136 - protein, 702 aa, artificial sequence
  Synthesized
QVQLKQSGPGLVQPSQSLSITCTVSGFSLTNYGVHWVRQSPGKGLEWLGVIWSGGNTDYNTPFTSRLSINKDNSKSQVFFKMNSLQSNDTAIYYCARALTYYDYEFAYWGQGTLVTVSSASTKGPSVFPLAPSSKSTSGGTAALGCLVKDYFPEPVTVSWNSGALTSGVHTFPAVLQSSGLYSLSSVVTVPSSSLGTQTYICNVNHKPSNTKVDKRVEPKSCDKTHTCPPCPAPELLGGPSVFLFPPKPKDTLMISRTPEVTCVVVDVSHEDPEVKFNWYVDGVEVHNAKTKPREEQYNSTYRVVSVLTVLHQDWLNGKEYKCKVSNKALPAPIEKTISKAKGQPREPQVYTLPPSRDELTKNQVSLTCLVKGFYPSDIAVEWESNGQPENNYKTTPPVLDSDGSFFLYSKLTVDKSRWQQGNVFSCSVMHEALHNHYTQKSLSLSPGGGGGSGGGGSQVQLQESGGGLVKPGGSLRLSCAASGFTFSSYWMSWVRQAPGKGLEWVANINRDGSASYYVDSVKGRFTISRDDAKNSLYLQMNSLRAEDTAVYYCARDRGVGYFDLWGRGTLVTVSSGGGGSGGGGSGGGGSQSALTQPASVSGSPGQSITISCTGTSSDVGGYNFVSWYQQHPGKAPKLMIYDVSDRPSGVSDRFSGSKSGNTASLIISGLQADDEADYYCSSYGSSSTHVIFGGGTKVTVL

SEQ ID NO: 137 - protein, 119 aa, artificial sequence; identical to SEQ ID NO: 48
  Synthesized

SEQ ID NO: 138 - protein, 244 aa, artificial sequence; identical to SEQ ID NO: 88
  Synthesized